European Patent Specification EP 4 153 232 B1, published June 26, 2024. Title: TNFalpha immunoconjugate therapy for the treatment of brain tumors. Applicant: Philogen S.p.A. The sequence listing filed with the application follows.

SEQUENCE LISTING (13 sequences)

SEQ ID NO: 1 - protein, 5 aa, Artificial Sequence
  synthetic construct
SFSMS

SEQ ID NO: 2 - protein, 17 aa, Artificial Sequence
  synthetic construct
SISGSSGTTYYADSVKG

SEQ ID NO: 3 - protein, 7 aa, Artificial Sequence
  synthetic construct
PFPYFDY

SEQ ID NO: 4 - protein, 12 aa, Artificial Sequence
  synthetic construct
RASQSVSSSFLA

SEQ ID NO: 5 - protein, 7 aa, Artificial Sequence
  synthetic construct
YASSRAT

SEQ ID NO: 6 - protein, 9 aa, Artificial Sequence
  synthetic construct
QQTGRIPPT

SEQ ID NO: 7 - protein, 116 aa, Artificial Sequence [sequence omitted]

SEQ ID NO: 8 - protein, 12 aa, Artificial Sequence
  synthetic construct
GDGSSGGSGGAS

SEQ ID NO: 9 - protein, 108 aa, Artificial Sequence [sequence omitted]

SEQ ID NO: 10 - protein, 236 aa, Artificial Sequence
  synthetic construct
EVQLLESGGGLVQPGGSLRLSCAASGFTFSSFSMSWVRQAPGKGLEWVSSISGSSGTTYYADSVKGRFTISRDNSKNTLYLQMNSLRAEDTAVYYCAKPFPYFDYWGQGTLVTVSSGDGSSGGSGGASEIVLTQSPGTLSLSPGERATLSCRASQSVSSSFLAWYQQKPGQAPRLLIYYASSRATGIPDRFSGSGSGTDFTLTISRLEPEDFAVYYCQQTGRIPPTFGQGTKVEIK

SEQ ID NO: 11 - protein, 157 aa, Artificial Sequence [sequence omitted]

SEQ ID NO: 12 - protein, 17 aa, Artificial Sequence
  synthetic construct
EFSSSSGSSSSGSSSSG

SEQ ID NO: 13 - protein, 410 aa, Artificial Sequence
  synthetic construct
EVQLLESGGGLVQPGGSLRLSCAASGFTFSSFSMSWVRQAPGKGLEWVSSISGSSGTTYYADSVKGRFTISRDNSKNTLYLQMNSLRAEDTAVYYCAKPFPYFDYWGQGTLVTVSSGDGSSGGSGGASEIVLTQSPGTLSLSPGERATLSCRASQSVSSSFLAWYQQKPGQAPRLLIYYASSRATGIPDRFSGSGSGTDFTLTISRLEPEDFAVYYCQQTGRIPPTFGQGTKVEIKEFSSSSGSSSSGSSSSGVRSSSRTPSDKPVAHVVANPQAEGQLQWLNRRANALLANGVELRDNQLVVPSEGLYLIYSQVLFKGQGCPSTHVLLTHTISRIAVSYQTKVNLLSAIKSPCQRETPEGAEAKPWYEPIYLGGVFQLEKGDRLSAEINRPDYLDFAESGQVYFGIIAL